European Patent Application EP 4 163 303 A1, published April 12, 2023. Title: SYNTHETIC MULTI-EPITOPE CHIMERA AS A VACCINE AND TREATMENT FOR LEISHMANIASIS IN MAMMALS. Applicant: Universidad Complutense de Madrid (UCM). The sequence listing filed with the application follows.

SEQUENCE LISTING (5 sequences)

SEQ ID NO: 1 - protein, 15 aa, Leishmania infantum
TAVLEYLTAELLELS

SEQ ID NO: 2 - protein, 24 aa, Leishmania infantum
RSLKAINAQMSMSHRTMKIVNSYV

SEQ ID NO: 3 - protein, 15 aa, Leishmania infantum
EGLRFQSSAIMALQE

SEQ ID NO: 4 - protein, 16 aa, Leishmania infantum
ITRGCVRRMARRGGVK

SEQ ID NO: 5 - protein, 70 aa, Artificial Sequence
  Multi-epitopic chimera consisting of SEQ ID NO: 1, 2, 3 and 4 from Leishmania infantum
TAVLEYLTAELLELSRSLKAINAQMSMSHRTMKIVNSYVEGLRFQSSAIMALQEITRGCVRRMARRGGVK